European Patent Application EP 4 303 322 A1, published January 10, 2024. Title: PRIMER-PROBE COMPOSITION, KIT, AND DETECTION METHOD. Applicant: ASCENTAWITS PHARMACEUTICALS, LTD. Application EP21928566.5. The sequence listing filed with the application follows.

SEQUENCE LISTING (19 sequences)

SEQ ID NO: 1 - DNA, 28 bp, Artificial Sequence
  AKR1C3-F1
ctcaacaagccaggactcaagtacaagc

SEQ ID NO: 2 - DNA, 32 bp, Artificial Sequence
  AKR1C3-R1
acttgcagaaatctagcaatttactccggttg

SEQ ID NO: 3 - DNA, 21 bp, Artificial Sequence
  AKR1C3-P1
ctgcaaccaggtagaatgtca

SEQ ID NO: 4 - DNA, 22 bp, Artificial Sequence
  AKR1C3-F2
acaagccaggactcaagtacaa

SEQ ID NO: 5 - DNA, 29 bp, Artificial Sequence
  AKR1C3-R2
aatctagcaatttactccggttgaaatac

SEQ ID NO: 6 - DNA, 27 bp, Artificial Sequence
  AKR1C3-R6
acttgcagaaatctagcaatttactcc

SEQ ID NO: 7 - DNA, 22 bp, Artificial Sequence
  AKR1C3-F6
gatgatcctcaacaagccagga

SEQ ID NO: 8 - DNA, 22 bp, Artificial Sequence
  AKR1C3-F5
tggcagtgtgaagagagragac

SEQ ID NO: 9 - DNA, 23 bp, Artificial Sequence
  AKR1C3-R5
ggtcaacatagtccaattgagct

SEQ ID NO: 10 - DNA, 22 bp, Artificial Sequence
  AKR1C3-P2
ctttggtccacttttcatcgac

SEQ ID NO: 11 - DNA, 29 bp, Artificial Sequence
  AKR1C3-F3
cagtgtgaagagagaagacatattctaca

SEQ ID NO: 12 - DNA, 18 bp, Artificial Sequence
  AKR1C3-R3
caaggctggtcggaccaa

SEQ ID NO: 13 - DNA, 20 bp, Artificial Sequence
  AKR1C3-F4
gcagatggcagtgtgaagag

SEQ ID NO: 14 - DNA, 27 bp, Artificial Sequence
  AKR1C3-F7
caccaacagatgaaaatggaaaagtaa

SEQ ID NO: 15 - DNA, 21 bp, Artificial Sequence
  AKR1C3-R7
ggttgaagtttgacaccccaa

SEQ ID NO: 16 - DNA, 24 bp, Artificial Sequence
  AKR1C3-P3
ttgacatagtggatctctgtacca

SEQ ID NO: 17 - DNA, 21 bp, Artificial Sequence
  ACTB-F1
caccttctacaatgagctgcg

SEQ ID NO: 18 - DNA, 24 bp, Artificial Sequence
  ACTB-R1
gtctcaaacatgatctgggtcatc

SEQ ID NO: 19 - DNA, 21 bp, Artificial Sequence
  ACTB-P1
cctcggtcagcagcacggggt